European Patent Application EP 4 134 430 A1, published February 15, 2023. Title: METHODS FOR ENHANCING EFFICACY OF THERAPEUTIC IMMUNE CELLS. Applicant: National University of Singapore CAMPANA, Dario KAMIYA, Takahiro. Application PCT/SG2016/050063. The sequence listing filed with the application follows.

SEQUENCE LISTING (64 sequences)

SEQ ID NO: 1 - protein, 10 aa, Artificial Sequence
  Myc tag
EQKLISEEDL

SEQ ID NO: 2 - DNA, 40 bp, Artificial Sequence
  Sense primer
atatatgaattcggcttccaccatggccttaccagtgacc

SEQ ID NO: 3 - DNA, 50 bp, Artificial Sequence
  Reverse primer
cagatcttcttcagaaataagtttttgttcggctgaggagactgtgagag

SEQ ID NO: 4 - protein, 4 aa, Artificial Sequence
  KDEL coding sequence
KDEL

SEQ ID NO: 5 - DNA, 40 bp, Artificial Sequence; identical to SEQ ID NO: 2
  Sense primer

SEQ ID NO: 6 - DNA, 48 bp, Artificial Sequence
  Reverse primer
tatatactcgagttacaactcgtccttcagatcttcttcagaaataag

SEQ ID NO: 7 - protein, 40 aa, Artificial Sequence
  PEST motif
SHGFPPEVEEQDDGTLPMSCAQESGMDRHPAACASARINV

SEQ ID NO: 8 - protein, 5 aa, Artificial Sequence
  Hydrophilic peptide
GGGGS

SEQ ID NO: 9 - protein, 4 aa, Artificial Sequence
  ER or Golgi retention sequence
  VARIANT 3, 4: Xaa = Any Amino Acid
KKXX

SEQ ID NO: 10 - protein, 3 aa, Artificial Sequence
  ER or Golgi retention sequence
  VARIANT 2: Xaa = Any Amino Acid
  VARIANT 3: Xaa = ASP or GLU
KXX

SEQ ID NO: 11 - protein, 4 aa, Artificial Sequence
  ER or Golgi retention sequence
YQRL

SEQ ID NO: 12 - protein, 120 aa, Artificial Sequence
  Variable heavy region for scFv targeting CD3
EVQLQQSGAELARPGASVKMSCKASGYTFTRYTMHWVKQRPGQGLEWIGYINPSRGYTNYNQKFKDKATLTTDKSSSTAYMQLSSLTSEDSAVYYCARYYDDHYCLDYWGQGTTLTVSSA

SEQ ID NO: 13 - protein, 107 aa, Artificial Sequence
  Variable light region for scFv targeting CD3
QIVLTQSPAIMSASPGEKVTMTCSASSSVSYMNWYQQKSGTSPKRWIYDTSKLASGVPAHFRGSGSGTSYSLTISGMEAEDAATYYCQQWSSNPFTFGSGTKLEINR

SEQ ID NO: 14 - DNA, 360 bp, Artificial Sequence
  Variable heavy region for scFv targeting CD3
gaggtccagctgcagcagtctggggctgaactggcaagacctggggcctcagtgaagatgtcctgcaaggcttctggctacacctttactaggtacacgatgcactgggtaaaacagaggcctggacagggtctggaatggattggatacattaatcctagccgtggttatactaattacaatcagaagttcaaggacaaggccacattgactacagacaaatcctccagcacagcctacatgcaactgagcagcctgacatctgaggactctgcagtctattactgtgcaagatattatgatgatcattactgccttgactactggggccaaggcaccactctcacagtctcctcagcc

SEQ ID NO: 15 - DNA, 321 bp, Artificial Sequence
  Variable light region for scFv targeting CD3
caaattgttctcacccagtctccagcaatcatgtctgcatctccaggggagaaggtcaccatgacctgcagtgccagctcaagtgtaagttacatgaactggtaccagcagaagtcaggcacctcccccaaaagatggatttatgacacatccaaactggcttctggagtccctgctcacttcaggggcagtgggtctgggacctcttactctctcacaatcagcggcatggaggctgaagatgctgccacttattactgccagcagtggagtagtaacccattcacgttcggctcggggacaaagttggaaataaaccgg

SEQ ID NO: 16 - protein, 117 aa, Artificial Sequence
  Variable heavy region for scFv targeting CD7 (TH69)
EVQLVESGGGLVKPGGSLKLSCAASGLTFSSYAMSWVRQTPEKRLEWVASISSGGFTYYPDSVKGRFTISRDNARNILYLQMSSLRSEDTAMYYCARDEVRGYLDVWGAGTTVTVSS

SEQ ID NO: 17 - protein, 112 aa, Artificial Sequence
  Variable light region for scFv targeting CD7 (TH69)
AAYKDIQMTQTTSSLSASLGDRVTISCSASQGISNYLNWYQQKPDGTVKLLIYYTSSLHSGVPSRFSGSGSGTDYSLTISNLEPEDIATYYCQQYSKLPYTFGGGTKLEIKR

SEQ ID NO: 18 - DNA, 351 bp, Artificial Sequence
  Variable heavy region for scFv targeting CD7 (TH69)
gaggtgcagctggtcgaatctggaggaggactggtgaagccaggaggatctctgaaactgagttgtgccgcttcaggcctgaccttctcaagctacgccatgagctgggtgcgacagacacctgagaagcggctggaatgggtcgctagcatctcctctggcgggttcacatactatccagactccgtgaaaggcagatttactatctctcgggataacgcaagaaatattctgtacctgcagatgagttcactgaggagcgaggacaccgcaatgtactattgtgccagggacgaagtgcgcggctatctggatgtctggggagctggcactaccgtcaccgtctccagc

SEQ ID NO: 19 - DNA, 336 bp, Artificial Sequence
  Variable light region for scFv targeting CD7 (TH69)
gccgcatacaaggatattcagatgactcagaccacaagctccctgagcgcctccctgggagaccgagtgacaatctcttgcagtgcatcacagggaattagcaactacctgaattggtatcagcagaagccagatggcactgtgaaactgctgatctactatacctctagtctgcacagtggggtcccctcacgattcagcggatccggctctgggacagactacagcctgactatctccaacctggagcccgaagatattgccacctactattgccagcagtactccaagctgccttatacctttggcgggggaacaaagctggagattaaaagg

SEQ ID NO: 20 - protein, 123 aa, Artificial Sequence
  Variable heavy region for scFv targeting CD7 (3a1f)
QVQLQESGAELVKPGASVKLSCKASGYTFTSYWMHWVKQRPGQGLEWIGKINPSNGRTNYNEKFKSKATLTVDKSSSTAYMQLSSLTSEDSAVYYCARGGVYYDLYYYALDYWGQGTTVTVSS

SEQ ID NO: 21 - protein, 108 aa, Artificial Sequence
  Variable light region for scFv targeting CD7 (3a1f)
DIELTQSPATLSVTPGDSVSLSCRASQSISNNLHWYQQKSHESPRLLIKSASQSISGIPSRFSGSGSGTDFTLSINSVETEDFGMYFCQQSNSWPYTFGGGTKLEIKR

SEQ ID NO: 22 - DNA, 369 bp, Artificial Sequence
  Variable heavy region for scFv targeting CD7 (3a1f)
caggtccagctgcaggagtcaggggcagagctggtgaaacccggagccagtgtcaaactgtcctgtaaggccagcggctatactttcaccagctactggatgcactgggtgaaacagaggccaggacagggcctggagtggatcggcaagattaaccccagcaatgggcgcaccaactacaacgaaaagtttaaatccaaggctacactgactgtggacaagagctcctctaccgcatacatgcagctgagttcactgacatctgaagatagtgccgtgtactattgcgccagaggcggggtctactatgacctgtactattacgcactggattattgggggcagggaaccacagtgactgtcagctcc

SEQ ID NO: 23 - DNA, 324 bp, Artificial Sequence
  Variable light region for scFv targeting CD7 (3a1f)
gacatcgagctgacacagtctccagccactctgagcgtgacccctggcgattctgtcagtctgtcatgtagagctagccagtccatctctaacaatctgcactggtaccagcagaaatcacatgaaagccctcggctgctgattaagagtgcttcacagagcatctccgggattccaagcagattctctggcagtgggtcaggaaccgactttacactgtccattaactctgtggagaccgaagatttcggcatgtatttttgccagcagagcaattcctggccttacacattcggaggcgggactaaactggagattaagagg

SEQ ID NO: 24 - protein, 120 aa, Artificial Sequence
  Variable heavy region for scFv targeting CD45
QVQLVESGGGLVQPGGSLKLSCAASGFDFSRYWMSWVRQAPGKGLEWIGEINPTSSTINFTPSLKDKVFISRDNAKNTLYLQMSKVRSEDTALYYCARGNYYRYGDAMDYWGQGTSVTVS

SEQ ID NO: 25 - protein, 111 aa, Artificial Sequence
  Variable light region for scFv targeting CD45
DIVLTQSPASLAVSLGQRATISCRASKSVSTSGYSYLHWYQQKPGQPPKLLIYLASNLESGVPARFSGSGSGTDFTLNIHPVEEEDAATYYCQHSRELPFTFGSGTKLEIK

SEQ ID NO: 26 - DNA, 360 bp, Artificial Sequence
  Variable heavy region for scFv targeting CD45
caggtgcagctggtcgagtctggaggaggactggtgcagcctggaggaagtctgaagctgtcatgtgcagccagcgggttcgacttttctcgatactggatgagttgggtgcggcaggcaccaggaaaaggactggaatggatcggcgagattaacccaactagctccaccatcaatttcacacccagcctgaaggacaaagtgtttatttccagagataacgccaagaatactctgtatctgcagatgtccaaagtcaggtctgaagataccgccctgtactattgtgctcggggcaactactatagatacggggacgctatggattattgggggcagggaactagcgtgaccgtgagt

SEQ ID NO: 27 - DNA, 333 bp, Artificial Sequence
  Variable light region for scFv targeting CD45
gacattgtgctgacccagtcccctgcttcactggcagtgagcctgggacagagggcaaccatcagctgccgagcctctaagagtgtctcaacaagcggatactcctatctgcactggtaccagcagaagccaggacagccacctaaactgctgatctatctggcttccaacctggaatctggagtgcctgcacgcttctccggatctggaagtggaaccgactttacactgaatattcacccagtcgaggaagaggatgccgctacctactattgccagcacagccgggagctgcccttcacatttggcagcgggactaagctggagatcaag

SEQ ID NO: 28 - protein, 119 aa, Artificial Sequence
  Variable heavy region for scFv targeting B2MG
EVQLQQSGAELVKPGASVKLSCTPSGFNVKDTYIHWVKQRPKQGLEWIGRIDPSDGDIKYDPKFQGKATITADTSSNTVSLQLSSLTSEDTAVYYCARWFGDYGAMNYWGQGTSVTVSS

SEQ ID NO: 29 - protein, 110 aa, Artificial Sequence
  Variable light region for scFv targeting B2MG
DIQMTQSPASQSASLGESVTITCLASQTIGTWLAWYQQKPGKSPQLLIYAATSLADGVPSRFSGSGSGTKFSLKIRTLQAEDFVSYYCQQLYSKPYTFGGGTKLEIKRAD

SEQ ID NO: 30 - DNA, 357 bp, Artificial Sequence
  Variable heavy region for scFv targeting B2MG
gaggtgcagctgcagcagagcggagcagaactggtgaaacctggagccagcgtcaagctgtcctgtactccatctggcttcaacgtgaaggacacatacattcactgggtcaagcagcggcccaaacagggactggagtggatcggcagaattgacccatccgacggcgatatcaagtatgatcccaaattccaggggaaggctactattaccgcagataccagctccaacacagtgagtctgcagctgtctagtctgactagcgaagacaccgccgtctactattgtgctagatggtttggcgattacggggccatgaattattgggggcagggaaccagcgtcaccgtgtccagc

SEQ ID NO: 31 - DNA, 330 bp, Artificial Sequence
  Variable light region for scFv targeting B2MG
gatattcagatgacccagtcccctgcatcacagagcgcctccctgggcgagtcagtgaccatcacatgcctggctagccagacaattggcacttggctggcatggtaccagcagaagcccggcaaatcccctcagctgctgatctatgcagctacctctctggcagacggagtgcccagtaggttctctgggagtggatcaggcaccaagttttctctgaaaattcgcacactgcaggctgaggatttcgtctcctactattgccagcagctgtactctaaaccttatacatttggcgggggaactaagctggaaatcaaacgagcagac

SEQ ID NO: 32 - protein, 119 aa, Artificial Sequence
  Variable heavy region for scFv targeting NKG2A
EVQLVESGGGLVKPGGSLKLSCAASGFTFSSYAMSWVRQSPEKRLEWVAEISSGGSYTYYPDTVTGRFTISRDNAKNTLYLEISSLRSEDTAMYYCTRHGDYPRFFDVWGAGTTVTVSS

SEQ ID NO: 33 - protein, 107 aa, Artificial Sequence
  Variable light region for scFv targeting NKG2A
QIVLTQSPALMSASPGEKVTMTCSASSSVSYIYWYQQKPRSSPKPWIYLTSNLASGVPARFSGSGSGTSYSLTISSMEAEDAATYYCQQWSGNPYTFGGGTKLEIKR

SEQ ID NO: 34 - DNA, 357 bp, Artificial Sequence
  Variable heavy region for scFv targeting NKG2A
gaggtgcagctggtggagagcggaggaggactggtgaagccaggaggaagcctgaagctgtcctgtgccgcctctggcttcacattttcctcttatgcaatgagctgggtgcggcagtccccagagaagagactggagtgggtggcagagatcagctccggaggatcctacacctactatcctgacacagtgaccggccggttcacaatctctagagataacgccaagaataccctgtatctggagatctctagcctgagatccgaggatacagccatgtactattgcaccaggcacggcgactacccacgcttctttgacgtgtggggagcaggaaccacagtgaccgtgtcctct

SEQ ID NO: 35 - DNA, 321 bp, Artificial Sequence
  Variable light region for scFv targeting NKG2A
cagattgtcctgacccagtctccagccctgatgagcgcctcccctggcgagaaggtgacaatgacctgctctgccagctcctctgtgagctacatctattggtaccagcagaagcctcggagctccccaaagccctggatctatctgacatccaacctggcctctggcgtgccagccagattctctggcagcggctccggcacatcttacagcctgaccatctctagcatggaggccgaggacgccgccacctactattgccagcagtggtccggcaatccatatacatttggcggcggcaccaagctggagatcaagagg

SEQ ID NO: 36 - protein, 122 aa, Artificial Sequence
  Variable heavy region for scFv targeting KIR2DL1 and 2/3
QVQLVQSGAEVKKPGSSVKVSCKASGGTFSFYAISWVRQAPGQGLEWMGGFIPIFGAANYAQKFQGRVTITADESTSTAYMELSSLRSDDTAVYYCARPSGSYYYDYDMDVWGQGTTVTVSS

SEQ ID NO: 37 - protein, 109 aa, Artificial Sequence
  Variable light region for scFv targeting KIR2DL1 and 2/3
EIVLTQSPVTLSLSPGERATLSCRASQSVSSYLAWYQQKPGQAPRLLIYDASNRATGIPARFSGSGSGTDFTLTISSLEPEDFAVYYCQQRSNWMYTFGQGTKLEIKRT

SEQ ID NO: 38 - DNA, 369 bp, Artificial Sequence
  Variable heavy region for scFv targeting KIR2DL1 and 2/3
caggtccagctggtgcagtctggagctgaagtgaagaaaccagggagctccgtcaaggtgtcatgcaaagcaagcggcgggactttctccttttatgcaatctcttgggtgagacaggcacctggacagggactggagtggatgggaggcttcatcccaatttttggagccgctaactatgcccagaagttccagggcagggtgaccatcacagctgatgagtctactagtaccgcatacatggaactgtctagtctgaggagcgacgataccgccgtgtactattgtgctcgcattccatcaggcagctactattacgactatgatatggacgtgtggggccaggggaccacagtcaccgtgagcagc

SEQ ID NO: 39 - DNA, 327 bp, Artificial Sequence
  Variable light region for scFv targeting KIR2DL1 and 2/3
gagatcgtgctgacccagtctcctgtcacactgagtctgtcaccaggggaacgggctacactgtcttgcagagcaagccagtccgtgagctcctacctggcctggtatcagcagaagccaggccaggctcccaggctgctgatctacgatgcaagcaacagggccactgggattcccgcccgcttctctggcagtgggtcaggaaccgactttactctgaccatttctagtctggagcctgaagatttcgccgtgtactattgccagcagcgatccaattggatgtatacttttggccaggggaccaagctggagatcaaacggaca

SEQ ID NO: 40 - protein, 21 aa, Artificial Sequence
  CD8 signal peptide
MALPVTALLLPLALLLHAARP

SEQ ID NO: 41 - protein, 20 aa, Artificial Sequence
  Variable heavy-variable light linker
GGGGSGGGGSGGGGSGGGGS

SEQ ID NO: 42 - protein, 70 aa, Artificial Sequence
  CD8 hinge and transmembrane
KPTTTPAPRPPTPAPTIASQPLSLRPEACRPAAGGAVHTRGLDFACDIYIWAPLAGTCGVLLLSLVITLY

SEQ ID NO: 43 - protein, 15 aa, Artificial Sequence
  Variable heavy-variable light linker
GGGGSGGGGSGGGGS

SEQ ID NO: 44 - DNA, 63 bp, Artificial Sequence
  CD8 signal peptide
atggccttaccagtgaccgccttgctcctgccgctggccttgctgctccacgccgccaggccg

SEQ ID NO: 45 - DNA, 63 bp, Artificial Sequence
  CD8 signal peptide
atggctctgcctgtgaccgcactgctgctgcccctggctctgctgctgcacgccgcaagacct

SEQ ID NO: 46 - DNA, 63 bp, Artificial Sequence
  CD8 signal peptide
atggctctgcccgtcaccgctctgctgctgcctctggctctgctgctgcacgctgctcgacca

SEQ ID NO: 47 - DNA, 63 bp, Artificial Sequence
  CD8 signal peptide
atggctctgcccgtgaccgctctgctgctgcctctggctctgctgctgcatgctgctcgacct

SEQ ID NO: 48 - DNA, 63 bp, Artificial Sequence
  CD8 signal peptide
atggccctgcccgtcaccgccctgctgctgcccctggctctgctgctgcacgccgcaagaccc

SEQ ID NO: 49 - DNA, 63 bp, Artificial Sequence
  CD8 signal peptide
atggctctgcccgtgaccgccctgctgctgcctctggctctgctgctgcacgctgcccgccca

SEQ ID NO: 50 - protein, 68 aa, Artificial Sequence
  CD8 hinge and transmembrane
TTTPAPRPPTPAPTIASQPLSLRPEACRPAAGGAVHTRGLDFACDIYIWAPLAGTCGVLLLSLVITLY

SEQ ID NO: 51 - DNA, 60 bp, Artificial Sequence
  Variable heavy-variable light linker
ggtggtggtggttctggtggtggtggttctggcggcggcggctccggtggtggtggatcc

SEQ ID NO: 52 - DNA, 60 bp, Artificial Sequence
  Variable heavy-variable light linker
ggaggaggaggaagcggaggaggaggatccggaggcgggggatctggaggaggaggaagt

SEQ ID NO: 53 - DNA, 45 bp, Artificial Sequence
  Variable heavy-variable light linker
ggaggaggaggatccggcggaggaggctctgggggaggcgggagt

SEQ ID NO: 54 - DNA, 60 bp, Artificial Sequence
  Variable heavy-variable light linker
ggaggaggaggaagtggaggaggaggatcaggaggcgggggaagcggcgggggaggctcc

SEQ ID NO: 55 - DNA, 60 bp, Artificial Sequence
  Variable heavy-variable light linker
ggaggaggaggaagtggaggaggagggtcaggaggcgggggaagcggcgggggaggatcc

SEQ ID NO: 56 - DNA, 60 bp, Artificial Sequence
  Variable heavy-variable light linker
ggaggaggaggatctggaggaggaggcagcggcggcggcggctccggcggcggcggctct

SEQ ID NO: 57 - DNA, 210 bp, Artificial Sequence
  CD8 hinge and transmembrane
aagcccaccacgacgccagcgccgcgaccaccaacaccggcgcccaccatcgcgtcgcagcccctgtccctgcgcccagaggcgtgccggccagcggcggggggcgcagtgcacacgagggggctggacttcgcctgtgatatctacatctgggcgcccttggccgggacttgtggggtccttctcctgtcactggttatcaccctttac

SEQ ID NO: 58 - DNA, 204 bp, Artificial Sequence
  CD8 hinge and transmembrane
accactacacctgcaccaaggcctcccacacccgctcccactatcgcttcccagccactgtccctgaggcccgaggcctgcaggccagcagctggcggagccgtgcatactagggggctggacttcgcttgcgacatctacatctgggccccactggcagggacatgcggagtcctgctgctgtccctggtcatcacactttac

SEQ ID NO: 59 - DNA, 204 bp, Artificial Sequence
  CD8 hinge and transmembrane
actaccacaccagctccaagaccacctacccctgcaccaacaattgctagtcagccactgtcactgagaccagaagcatgtaggcctgcagctggaggagctgtgcacaccagaggcctggactttgcctgcgatatctacatttgggctcctctggcaggaacctgtggcgtgctgctgctgtctctggtcatcacactttac

SEQ ID NO: 60 - DNA, 210 bp, Artificial Sequence
  CD8 hinge and transmembrane
aagccaaccacaacccctgcaccaaggccacctacaccagcacctaccatcgcaagccagccactgtccctgaggccagaggcatgtaggcctgcagcaggaggcgccgtgcacacacgcggcctggactttgcctgcgatatctacatctgggcaccactggcaggaacctgtggcgtgctgctgctgagcctggtgattaccctgtat

SEQ ID NO: 61 - DNA, 30 bp, Artificial Sequence
  Variable heavy-variable light linker
ggtggtggcggcagtggtggcggtggctca

SEQ ID NO: 62 - protein, 10 aa, Artificial Sequence
  Variable heavy-variable light linker
GGGGSGGGGS

SEQ ID NO: 63 - DNA, 60 bp, Artificial Sequence
  Variable heavy-variable light linker
ggtggtggcggcagtggtggcggtggctcaggcggtggtggctccggtggcggtggctct

SEQ ID NO: 64 - protein, 6 aa, Artificial Sequence
  Variable heavy-variable light linker
EEKKMP